European Patent Application EP 4 265 639 A2, published October 25, 2023. Title: Anti-HVEM antibodies, and compositions and methods related thereto. Applicant: Medytox Inc. The sequence listing filed with the application follows.

SEQUENCE LISTING (90 sequences)

SEQ ID NO: 1 - protein, 5 aa, Artificial Sequence
  HVEM011 HCDR1
SYAMH

SEQ ID NO: 2 - protein, 17 aa, Artificial Sequence
  HVEM011 HCDR2
SITSASSYIDYADSVKG

SEQ ID NO: 3 - protein, 8 aa, Artificial Sequence
  HVEM011 HCDR3
GTRGLFDH

SEQ ID NO: 4 - protein, 11 aa, Artificial Sequence
  HVEM011 LCDR1
RASRSVGKYLA

SEQ ID NO: 5 - protein, 7 aa, Artificial Sequence
  HVEM011 LCDR2
LGSNRAS

SEQ ID NO: 6 - protein, 10 aa, Artificial Sequence
  HVEM011 LCDR3
QQYGSSPPIT

SEQ ID NO: 7 - protein, 117 aa, Artificial Sequence
  HVEM011 VH
EVQLLESGGGLVQPGGSLRLSCAASEFTFSSYAMHWVRQAPGKGLEWVSSITSASSYIDYADSVKGRFTISRDNSKNTLYLQMNSLRAEDTAVYYCARGTRGLFDHWGQGTLVTVSS

SEQ ID NO: 8 - protein, 108 aa, Artificial Sequence
  HVEM011 VL
EIVLTQSPGTLSLSPGERATLSCRASRSVGKYLAWYQQKPGQAPRLLIYLGSNRASGIPDRFSGSGSGTDFTLTISRLEPEDFAVYYCQQYGSSPPITFGQGTKVEIK

SEQ ID NO: 9 - protein, 5 aa, Artificial Sequence
  HVEM021 HCDR1
TFAMH

SEQ ID NO: 10 - protein, 15 aa, Artificial Sequence
  HVEM021 HCDR2
SIYPSGNTHYKPSLK

SEQ ID NO: 11 - protein, 11 aa, Artificial Sequence
  HVEM021 HCDR3
RHPGGGWIFDY

SEQ ID NO: 12 - protein, 11 aa, Artificial Sequence
  HVEM021 LCDR1
RASRSVGKYLA

SEQ ID NO: 13 - protein, 7 aa, Artificial Sequence
  HVEM021 LCDR2
GASTRAT

SEQ ID NO: 14 - protein, 10 aa, Artificial Sequence
  HVEM021 LCDR3
QQYGSSPPVT

SEQ ID NO: 15 - protein, 119 aa, Artificial Sequence
  HVEM021 VH
EVQLLESGGGLVQPGGSLRLSCAASGFTFSTFAMHWVRQAPGKGLEWVSSIYPSGNTHYKPSLKSRFTISRDNSKNTLYLQMNSLRAEDTAVYYCARRHPGGGWIFDYWGQGTLVTVSS

SEQ ID NO: 16 - protein, 108 aa, Artificial Sequence
  HVEM021 VL
EIVLTQSPGTLSLSPGERATLSCRASRSVGKYLAWYQQKPGQAPRLLIYGASTRATGIPDRFSGSGSGTDFTLTISRLEPEDFAVYYCQQYGSSPPVTFGQGTKVEIK

SEQ ID NO: 17 - protein, 5 aa, Artificial Sequence
  HVEM001 HCDR1
NYAMH

SEQ ID NO: 18 - protein, 17 aa, Artificial Sequence
  HVEM001 HCDR2
NINPSGGSTTYAQEFED

SEQ ID NO: 19 - protein, 12 aa, Artificial Sequence
  HVEM001 HCDR3
RSRQDSWGYFDI

SEQ ID NO: 20 - protein, 11 aa, Artificial Sequence
  HVEM001 LCDR1
RASRSISNYLA

SEQ ID NO: 21 - protein, 7 aa, Artificial Sequence
  HVEM001 LCDR2
GASTRAT

SEQ ID NO: 22 - protein, 10 aa, Artificial Sequence
  HVEM001 LCDR3
QQYGSSPPLT

SEQ ID NO: 23 - protein, 121 aa, Artificial Sequence
  HVEM001 VH
EVQLLESGGGLVQPGGSLRLSCAASGFTFSNYAMHWVRQAPGKGLEWVSNINPSGGSTTYAQEFEDRFTISRDNSKNTLYLQMNSLRAEDTAVYYCATRSRQDSWGYFDIWGQGTLVTVSS

SEQ ID NO: 24 - protein, 108 aa, Artificial Sequence
  HVEM001 VL
EIVLTQSPGTLSLSPGERATLSCRASRSISNYLAWYQQKPGQAPRLLIYGASTRATGIPDRFSGSGSGTDFTLTISRLEPEDFAVYYCQQYGSSPPLTFGQGTKVEIK

SEQ ID NO: 25 - protein, 5 aa, Artificial Sequence
  HVEM004 HCDR1
SYAMS

SEQ ID NO: 26 - protein, 17 aa, Artificial Sequence
  HVEM004 HCDR2
SISGSGGKTYYADSVRG

SEQ ID NO: 27 - protein, 12 aa, Artificial Sequence
  HVEM004 HCDR3
GVGYTTSGRFDY

SEQ ID NO: 28 - protein, 11 aa, Artificial Sequence
  HVEM004 LCDR1
RASRSISSYLA

SEQ ID NO: 29 - protein, 7 aa, Artificial Sequence
  HVEM004 LCDR2
GVSTRAT

SEQ ID NO: 30 - protein, 10 aa, Artificial Sequence
  HVEM004 LCDR3
QQYGSWPPFT

SEQ ID NO: 31 - protein, 121 aa, Artificial Sequence
  HVEM004 VH
EVQLLESGGGLVQPGGSLRLSCAASGFTFSSYAMSWVRQAPGKGLEWVSSISGSGGKTYYADSVRGRFTISRDNSKNTLYLQMNSLRAEDTAVYYCAKGVGYTTSGRFDYWGQGTLVTVSS

SEQ ID NO: 32 - protein, 108 aa, Artificial Sequence
  HVEM004 VL
EIVLTQSPGTLSLSPGERATLSCRASRSISSYLAWYQQKPGQAPRLLIYGVSTRATGIPDRFSGSGSGTDFTLTISRLEPEDFAVYYCQQYGSWPPFTFGQGTKVEIK

SEQ ID NO: 33 - protein, 5 aa, Artificial Sequence
  HVEM017 HCDR1
TNYMS

SEQ ID NO: 34 - protein, 17 aa, Artificial Sequence
  HVEM017 HCDR2
LISYSGSNKYYADSVKG

SEQ ID NO: 35 - protein, 12 aa, Artificial Sequence
  HVEM017 HCDR3
GRGNTISGTFDL

SEQ ID NO: 36 - protein, 11 aa, Artificial Sequence
  HVEM017 LCDR1
RASRSVGKYLA

SEQ ID NO: 37 - protein, 7 aa, Artificial Sequence
  HVEM017 LCDR2
SASTLSS

SEQ ID NO: 38 - protein, 10 aa, Artificial Sequence
  HVEM017 LCDR3
QQYGSSPPIT

SEQ ID NO: 39 - protein, 121 aa, Artificial Sequence
  HVEM017 VH
EVQLLESGGGLVQPGGSLRLSCAASGFTFSTNYMSWVRQAPGKGLEWVSLISYSGSNKYYADSVKGRFTISHDNSKNTLYLQMNSLRAEDTAVYYCARGRGNTISGTFDLWGQGTLVTVSS

SEQ ID NO: 40 - protein, 108 aa, Artificial Sequence
  HVEM017 VL
EIVLTQSPGTLSLSPGERATLSCRASRSVGKYLAWYQQKPGQAPRLLIYSASTLSSGIPDRFSGSGSGTDFTLTISRLEPEDFAVYYCQQYGSSPPITFGQGTKVEIK

SEQ ID NO: 41 - protein, 5 aa, Artificial Sequence
  HVEM018 HCDR1
SYSMN

SEQ ID NO: 42 - protein, 17 aa, Artificial Sequence
  HVEM018 HCDR2
AISGSGGGTYSADSVKG

SEQ ID NO: 43 - protein, 9 aa, Artificial Sequence
  HVEM018 HCDR3
GKAYGYFDY

SEQ ID NO: 44 - protein, 11 aa, Artificial Sequence
  HVEM018 LCDR1
RASRSVGKYLA

SEQ ID NO: 45 - protein, 7 aa, Artificial Sequence
  HVEM018 LCDR2
AASTLQS

SEQ ID NO: 46 - protein, 10 aa, Artificial Sequence
  HVEM018 LCDR3
QQYGSSPPVI

SEQ ID NO: 47 - protein, 118 aa, Artificial Sequence
  HVEM018 VH
EVQLLESGGGLVQPGGSLRLSCAASGFTFSSYSMNWVRQAPGKGLEWVSAISGSGGGTYSADSVKGRFTISRDNSKNTLYLQMNSLRAEDTAVYYCARGKAYGYFDYWGQGTLVTVSS

SEQ ID NO: 48 - protein, 108 aa, Artificial Sequence
  HVEM018 VL
EIVLTQSPGTLSLSPGERATLSCRASRSVGKYLAWYQQKPGQAPRLLIYAASTLQSGIPDRFSGSGSGTDFTLTISRLEPEDFAVYYCQQYGSSPPVIFGQGTKVEIK

SEQ ID NO: 49 - protein, 5 aa, Artificial Sequence
  HVEM030 HCDR1
GYYWT

SEQ ID NO: 50 - protein, 17 aa, Artificial Sequence
  HVEM030 HCDR2
TISASGDSTYYADSVKG

SEQ ID NO: 51 - protein, 9 aa, Artificial Sequence
  HVEM030 HCDR3
DRTFGYFDY

SEQ ID NO: 52 - protein, 11 aa, Artificial Sequence
  HVEM030 LCDR1
RASRSVGKYLA

SEQ ID NO: 53 - protein, 7 aa, Artificial Sequence
  HVEM030 LCDR2
AASSLQS

SEQ ID NO: 54 - protein, 10 aa, Artificial Sequence
  HVEM030 LCDR3
QQYGSSPPIT

SEQ ID NO: 55 - protein, 118 aa, Artificial Sequence
  HVEM030 VH
EVQLLESGGGLVQPGGSLRLSCAASGFTFSGYYWTWVRQAPGKGLEWVSTISASGDSTYYADSVKGRFTISRDNSKNTLYLQMNSLRAEDTAVYYCAHDRTFGYFDYWGQGTLVTVSS

SEQ ID NO: 56 - protein, 108 aa, Artificial Sequence
  HVEM030 VL
EIVLTQSPGTLSLSPGERATLSCRASRSVGKYLAWYQQKPGQAPRLLIYAASSLQSGIPDRFSGSGSGTDFTLTISRLEPEDFAVYYCQQYGSSPPITFGQGTKVEIK

SEQ ID NO: 57 - protein, 5 aa, Artificial Sequence
  HVEM032 HCDR1
NYAIH

SEQ ID NO: 58 - protein, 17 aa, Artificial Sequence
  HVEM032 HCDR2
TISSPGSTINYADSVKG

SEQ ID NO: 59 - protein, 9 aa, Artificial Sequence
  HVEM032 HCDR3
GYLYPAMDV

SEQ ID NO: 60 - protein, 11 aa, Artificial Sequence
  HVEM032 LCDR1
RASRSVGKYLS

SEQ ID NO: 61 - protein, 7 aa, Artificial Sequence
  HVEM032 LCDR2
GASKLQS

SEQ ID NO: 62 - protein, 10 aa, Artificial Sequence
  HVEM032 LCDR3
QQYGSWPPFT

SEQ ID NO: 63 - protein, 118 aa, Artificial Sequence
  HVEM032 VH
EVQLLESGGGLVQPGGSLRLSCAASGFTFSNYAIHWVRQAPGKGLEWVSTISSPGSTINYADSVKGRFTISRDNSKNTLYLQMNSLRAEDTAVYYCASGYLYPAMDVWGQGTLVTVSS

SEQ ID NO: 64 - protein, 108 aa, Artificial Sequence
  HVEM032 VL
EIVLTQSPGTLSLSPGERATLSCRASRSVGKYLSWYQQKPGQAPRLLIYGASKLQSGIPDRFSGSGSGTDFTLTISRLEPEDFAVYYCQQYGSWPPFTFGQGTKVEIK

SEQ ID NO: 65 - protein, 5 aa, Artificial Sequence
  HVEM039 HCDR1
SYGMN

SEQ ID NO: 66 - protein, 17 aa, Artificial Sequence
  HVEM039 HCDR2
IINPSGDTTTYAQKFQG

SEQ ID NO: 67 - protein, 7 aa, Artificial Sequence
  HVEM039 HCDR3
GRGAFDY

SEQ ID NO: 68 - protein, 11 aa, Artificial Sequence
  HVEM039 LCDR1
RASRSVGKYLA

SEQ ID NO: 69 - protein, 7 aa, Artificial Sequence
  HVEM039 LCDR2
GATSRAT

SEQ ID NO: 70 - protein, 10 aa, Artificial Sequence
  HVEM039 LCDR3
QQYGSSPPVT

SEQ ID NO: 71 - protein, 116 aa, Artificial Sequence
  HVEM039 VH
EVQLLESGGGLVQPGGSLRLSCAASGFTFSSYGMNWVRQAPGKGLEWVSIINPSGDTTTYAQKFQGRFTISRDNSKNTLYLQMNSLRAEDTAVYYCARGRGAFDYWGQGTLVTVSS

SEQ ID NO: 72 - protein, 108 aa, Artificial Sequence
  HVEM039 VL
EIVLTQSPGTLSLSPGERATLSCRASRSVGKYLAWYQQKPGQAPRLLIYGATSRATGIPDRFSGSGSGTDFTLTISRLEPEDFAVYYCQQYGSSPPVTFGQGTKVEIK

SEQ ID NO: 73 - protein, 5 aa, Artificial Sequence
  HVEM040 HCDR1
NYGMS

SEQ ID NO: 74 - protein, 15 aa, Artificial Sequence
  HVEM040 HCDR2
SIYYSGDTYYNPSLE

SEQ ID NO: 75 - protein, 9 aa, Artificial Sequence
  HVEM040 HCDR3
ASGSNAFDI

SEQ ID NO: 76 - protein, 11 aa, Artificial Sequence
  HVEM040 LCDR1
RASRSVGKYLA

SEQ ID NO: 77 - protein, 7 aa, Artificial Sequence
  HVEM040 LCDR2
GASSRTT

SEQ ID NO: 78 - protein, 10 aa, Artificial Sequence
  HVEM040 LCDR3
QQYGSSPPVT

SEQ ID NO: 79 - protein, 115 aa, Artificial Sequence
  HVEM040 VH
EVQLLESGGGLVQPGGSLRLSCAASGFTFSNYGMSWVRQAPGKGLEWVSSIYYSGDTYYNPSLESRFTISRDNSKNTLYLQMNSLRAEDTAVYYCASGSNAFDIWGQGTLVTVSS

SEQ ID NO: 80 - protein, 108 aa, Artificial Sequence
  HVEM040 VL
EIVLTQSPGTLSLSPGERATLSCRASRSVGKYLAWYQQKPGQAPRLLIYGASSRTTGIPDRFSGSGSGTDFTLTISRLEPEDFAVYYCQQYGSSPPVTFGQGTKVEIK

SEQ ID NO: 81 - protein, 5 aa, Artificial Sequence
  HVEM041 HCDR1
SYAMS

SEQ ID NO: 82 - protein, 16 aa, Artificial Sequence
  HVEM041 HCDR2
EISQSGSSNYNPSLKS

SEQ ID NO: 83 - protein, 7 aa, Artificial Sequence
  HVEM041 HCDR3
GRWRFDY

SEQ ID NO: 84 - protein, 11 aa, Artificial Sequence
  HVEM041 LCDR1
RASRSVGKYLA

SEQ ID NO: 85 - protein, 7 aa, Artificial Sequence
  HVEM041 LCDR2
GASTRAT

SEQ ID NO: 86 - protein, 10 aa, Artificial Sequence
  HVEM041 LCDR3
QQYGSSPPVT

SEQ ID NO: 87 - protein, 115 aa, Artificial Sequence
  HVEM041 VH
EVQLLESGGGLVQPGGSLRLSCAASGFTFSSYAMSWVRQAPGKGLEWVSEISQSGSSNYNPSLKSRFTISRDNSKNTLYLQMNSLRAEDTAVYYCATGRWRFDYWGQGTLVTVSS

SEQ ID NO: 88 - protein, 108 aa, Artificial Sequence; identical to SEQ ID NO: 16
  HVEM041 VL

SEQ ID NO: 89 - protein, 327 aa, Artificial Sequence
  Human antibody CH
ASTKGPSVFPLAPCSRSTSESTAALGCLVKDYFPEPVTVSWNSGALTSGVHTFPAVLQSSGLYSLSSVVTVPSSSLGTKTYTCNVDHKPSNTKVDKRVESKYGPPCPPCPAPEFLGGPSVFLFPPKPKDTLMISRTPEVTCVVVDVSQEDPEVQFNWYVDGVEVHNAKTKPREEQFNSTYRVVSVLTVLHQDWLNGKEYKCKVSNKGLPSSIEKTISKAKGQPREPQVYTLPPSQEEMTKNQVSLTCLVKGFYPSDIAVEWESNGQPENNYKTTPPVLDSDGSFFLYSRLTVDKSRWQEGNVFSCSVMHEALHNHYTQKSLSLSLGK

SEQ ID NO: 90 - protein, 107 aa, Artificial Sequence [sequence omitted]